European Patent Application EP 4 613 775 A1, published September 10, 2025. Title: Tumor-specific antibody. Applicant: Eberhard Karls Universität Tübingen - Medizinische Fakultät. Application EP. The sequence listing filed with the application follows.

SEQUENCE LISTING (83 sequences)

SEQ ID NO: 1 - protein, 14 aa, synthetic construct
ARSRGIVGSTLDDN

SEQ ID NO: 2 - protein, 14 aa, synthetic construct
AHRPIASSRDGFDY

SEQ ID NO: 3 - protein, 11 aa, synthetic construct
SHHRLTDGRLR

SEQ ID NO: 4 - protein, 9 aa, synthetic construct
QQYHSTPRT

SEQ ID NO: 5 - protein, 9 aa, synthetic construct
QQYNGFPFT

SEQ ID NO: 6 - protein, 9 aa, synthetic construct
QQYDTSPWT

SEQ ID NO: 7 - protein, 8 aa, synthetic construct
ISVYKSDT

SEQ ID NO: 8 - protein, 7 aa, synthetic construct
IYWNDDK

SEQ ID NO: 9 - protein, 7 aa, synthetic construct
VYWDDDK

SEQ ID NO: 10-12 - skipped (3 entries)

SEQ ID NO: 13 - protein, 8 aa, synthetic construct
GYTFTSYG

SEQ ID NO: 14 - protein, 10 aa, synthetic construct
GFSLSTNGVS

SEQ ID NO: 15 - protein, 10 aa, synthetic construct
GFSLNTRAVG

SEQ ID NO: 16 - protein, 12 aa, synthetic construct
QSVLYSSNNRNY

SEQ ID NO: 17 - protein, 6 aa, synthetic construct
QSVSGW

SEQ ID NO: 18 - protein, 7 aa, synthetic construct
QSITSSY

SEQ ID NO: 19 - protein, 121 aa, synthetic construct
QVQLVESGPEVKKPGASVKVSCKASGYTFTSYGISWVRQAPGQGLEWMGWISVYKSDTNDAQKFQGRVTMTTDTSTSTAYMELRSLRSDDTAVYYCARSRGIVGSTLDDNWGQGTLVTVSS

SEQ ID NO: 20 - protein, 113 aa, synthetic construct
HPQMTQSPDSLAVSLGERATINCKSSQSVLYSSNNRNYLAWYQQKPGQPPKLLIYWASTRESGVPDRFSGSGSGTDFTLTISSLQAEDVAVYYCQQYHSTPRTFGQGTKVEIK

SEQ ID NO: 21 - protein, 122 aa, synthetic construct
QVPLKESGPALVKPTRTLTLTCTFSGFSLSTNGVSVGWIRQPPGKALDWLALIYWNDDKRYSPSLKNRLTITKDTSKNLVVLRMTNMDPVDTATYYCAHRPIASSRDGFDYWGQGTLVTVSS

SEQ ID NO: 22 - protein, 107 aa, synthetic construct
DIQMTQFPSTLSASVGETVTISCRASQSVSGWLAWYQQKPGKAPKLLMYKASALENGVPSRFSGSGSGTEFTLTISSLQPDDFATYYCQQYNGFPFTFGPGTKVDIN

SEQ ID NO: 23 - protein, 119 aa, synthetic construct
QVQLVESGPTLVKPTQTLTVTCTFSGFSLNTRAVGVGWIRQPPGGALEWLALVYWDDDKRYSPSLKNRLTITKDTSRNQVVLTLTNVAPVDTGTYYCSHHRLTDGRLRWGQGTLVTVSS

SEQ ID NO: 24 - protein, 108 aa, synthetic construct
QVQLVQSPGTLSLSPGERATLSCRASQSITSSYLAWYQQKFGQAPRLLIYRASNRATGIPDRFSGSGSGTDFTLTISSLESEDFAVYYCQQYDTSPWTFGQGTKVEIK

SEQ ID NO: 25 - DNA, 42 bp, synthetic construct
  source 1..42: mol_type = other DNA
gcccgctctaggggcatcgtgggcagtacactggacgacaac

SEQ ID NO: 26 - DNA, 42 bp, synthetic construct
  source 1..42: mol_type = other DNA
gcccacaggcccatcgcctcctcccgagacggcttcgactac

SEQ ID NO: 27 - DNA, 33 bp, synthetic construct
  source 1..33: mol_type = other DNA
agccaccacaggctgaccgacggaagactgagg

SEQ ID NO: 28 - DNA, 27 bp, synthetic construct
  source 1..27: mol_type = other DNA
cagcagtaccactccacccccagaacc

SEQ ID NO: 29 - DNA, 27 bp, synthetic construct
  source 1..27: mol_type = other DNA
cagcagtacaatggctttcccttcaca

SEQ ID NO: 30 - DNA, 27 bp, synthetic construct
  source 1..27: mol_type = other DNA
cagcagtacgacacctctccctggacc

SEQ ID NO: 31 - DNA, 24 bp, synthetic construct
  source 1..24: mol_type = other DNA
atctccgtgtataagagcgataca

SEQ ID NO: 32 - DNA, 21 bp, synthetic construct
  source 1..21: mol_type = other DNA
atctactggaacgacgacaaa

SEQ ID NO: 33 - DNA, 21 bp, synthetic construct
  source 1..21: mol_type = other DNA
gtgtactgggacgacgacaag

SEQ ID NO: 34-36 - skipped (3 entries)

SEQ ID NO: 37 - DNA, 24 bp, synthetic construct
  source 1..24: mol_type = other DNA
ggctacaccttcacctcctacggc

SEQ ID NO: 38 - DNA, 30 bp, synthetic construct
  source 1..30: mol_type = other DNA
ggcttctccctgtccaccaacggcgtgtcc

SEQ ID NO: 39 - DNA, 30 bp, synthetic construct
  source 1..30: mol_type = other DNA
ggcttctcactgaacacaagggccgtgggc

SEQ ID NO: 40 - DNA, 36 bp, synthetic construct
  source 1..36: mol_type = other DNA
cagtccgtcctctactcctccaacaaccgcaactac

SEQ ID NO: 41 - DNA, 18 bp, synthetic construct
  source 1..18: mol_type = other DNA
cagtccgtgtccggctgg

SEQ ID NO: 42 - DNA, 21 bp, synthetic construct
  source 1..21: mol_type = other DNA
cagtcaatcacatcctcctac

SEQ ID NO: 43 - DNA, 363 bp, synthetic construct
  source 1..363: mol_type = other DNA
caggtgcagctggtggaaagtggccccgaggtgaaaaagcccggcgcctccgtgaaggtgtcctgcaaagcaagcggctacaccttcacctcctacggcatctcctgggtgaggcaggcccccggacagggactggagtggatgggatggatctccgtgtataagagcgatacaaatgacgcccagaagttccagggccgcgtgacaatgaccaccgacacctccaccagcaccgcttatatggagctgagatccctgaggagcgacgacaccgccgtgtactactgtgcccgctctaggggcatcgtgggcagtacactggacgacaactggggccagggcaccctggtgacagtgagctcc

SEQ ID NO: 44 - DNA, 339 bp, synthetic construct
  source 1..339: mol_type = other DNA
caccctcagatgacccagtcccccgactccctggccgtctccctcggagaaagagccaccatcaactgcaaatcctcccagtccgtcctctactcctccaacaaccgcaactacctcgcctggtaccagcagaaacccggccagccccccaaactgctcatctactgggcatccaccagagaatccggcgtgcccgaccgcttctccggctctggaagcggcaccgacttcaccctgactatctcctccctgcaggctgaggacgtcgccgtttactactgccagcagtaccactccacccccagaaccttcggccagggcaccaaggtggaaatcaaa

SEQ ID NO: 45 - DNA, 366 bp, synthetic construct
  source 1..366: mol_type = other DNA
caggtgccactgaaggaaagcggccccgccctggtgaaacccaccagaacactgaccctgacctgcaccttctccggcttctccctgtccaccaacggcgtgtccgtgggctggatcaggcagccccccggaaaagccctggactggctggctctgatctactggaacgacgacaaaagatactccccctccctgaagaaccggctgaccatcacaaaagacaccagcaagaacctggtggtgctgaggatgaccaacatggaccctgtggacaccgccacctactactgcgcccacaggcccatcgcctcctcccgagacggcttcgactactggggacagggaaccctggtgaccgtgtccagc

SEQ ID NO: 46 - DNA, 321 bp, synthetic construct
  source 1..321: mol_type = other DNA
gacattcagatgacccagtttccctccaccctgtccgcctccgtgggcgaaaccgtgaccatctcctgcagggcctcccagtccgtgtccggctggctggcttggtaccagcagaaacccggcaaagcccccaaactgctgatgtacaaagcctccgccctggagaacggcgtgccctcacgctttagcggttccggctccgggaccgagttcaccctgactatctcctcactgcagcccgacgacttcgccacctactactgccagcagtacaatggctttcccttcacattcggtcccggcacaaaggtggatattaac

SEQ ID NO: 47 - DNA, 357 bp, synthetic construct
  source 1..357: mol_type = other DNA
caggtgcagctggtggaaagtggccccaccctggtgaagcccacacagacactgacagtgacatgcacattctccggcttctcactgaacacaagggccgtgggcgtgggatggatcaggcagccccccggaggcgcactggaatggctggctctggtgtactgggacgacgacaagaggtactcccctagtctgaagaacaggctgacaatcacaaaggataccagcaggaaccaggtggtgctgacactgaccaacgtggctcccgtggacaccggcacctactactgcagccaccacaggctgaccgacggaagactgaggtggggccagggcaccctggtgacagtgtcctct

SEQ ID NO: 48 - DNA, 324 bp, synthetic construct
  source 1..324: mol_type = other DNA
caggtccagctcgtccagagccccggcacactctccctctcccccggagaaagagccacactctcatgccgggcctcccagtcaatcacatcctcctacctcgcctggtaccagcagaaattcggccaggcccccaggctcctgatctacagggcctccaacagggccaccggaatccccgacaggttttccggctccggctccggaaccgacttcaccctgactatctcctccctcgagtctgaggacttcgcagtttactactgccagcagtacgacacctctccctggaccttcggccagggtaccaaggtggagatcaag

SEQ ID NO: 49 - protein, 11 aa, synthetic construct
RIFGNREMKAK

SEQ ID NO: 50 - protein, 13 aa, synthetic construct
SGEKRLIPKPTCR

SEQ ID NO: 51 - protein, 5 aa, synthetic construct
HVYNY

SEQ ID NO: 52 - protein, 11 aa, synthetic construct
EYTITVSAAEI

SEQ ID NO: 53 - protein, 11 aa, synthetic construct
SWSSQEHLEWE

SEQ ID NO: 54 - protein, 7 aa, synthetic construct
LEYLDLY

SEQ ID NO: 55 - protein, 7 aa, synthetic construct
TVDGKRV

SEQ ID NO: 56 - protein, 15 aa, synthetic construct
EAKVRIFGNREMKAK

SEQ ID NO: 57 - protein, 15 aa, synthetic construct
KVRIFGNREMKAKAK

SEQ ID NO: 58 - protein, 15 aa, synthetic construct
RIFGNREMKAKAKAA

SEQ ID NO: 59 - protein, 15 aa, synthetic construct
LKSGEKRLIPKPTCR

SEQ ID NO: 60 - protein, 15 aa, synthetic construct
SGEKRLIPKPTCRFK

SEQ ID NO: 61 - protein, 15 aa, synthetic construct
SRGLDLNDVTHVYNY

SEQ ID NO: 62 - protein, 15 aa, synthetic construct
GLDLNDVTHVYNYDF

SEQ ID NO: 63 - protein, 15 aa, synthetic construct
HVYNYDFPRNIDVYV

SEQ ID NO: 64 - protein, 15 aa, synthetic construct
ASDWEYTITVSAAEI

SEQ ID NO: 65 - protein, 15 aa, synthetic construct
DWEYTITVSAAEIYN

SEQ ID NO: 66 - protein, 15 aa, synthetic construct
EYTITVSAAEIYNEV

SEQ ID NO: 67 - protein, 15 aa, synthetic construct
AELGSWSSQEHLEWE

SEQ ID NO: 68 - protein, 15 aa, synthetic construct
LGSWSSQEHLEWEPA

SEQ ID NO: 69 - protein, 15 aa, synthetic construct
SWSSQEHLEWEPACQ

SEQ ID NO: 70 - protein, 15 aa, synthetic construct
RKTLADLQLEYLDLY

SEQ ID NO: 71 - protein, 15 aa, synthetic construct
TLADLQLEYLDLYLM

SEQ ID NO: 72 - protein, 15 aa, synthetic construct
ADLQLEYLDLYLMHW

SEQ ID NO: 73 - protein, 15 aa, synthetic construct
LQLEYLDLYLMHWPY

SEQ ID NO: 74 - protein, 15 aa, synthetic construct
LEYLDLYLMHWPYAF

SEQ ID NO: 75 - protein, 15 aa, synthetic construct
WRYIVPMLTVDGKRV

SEQ ID NO: 76 - protein, 15 aa, synthetic construct
YIVPMLTVDGKRVPR

SEQ ID NO: 77 - protein, 15 aa, synthetic construct
VPMLTVDGKRVPRDA

SEQ ID NO: 78 - protein, 15 aa, synthetic construct
MLTVDGKRVPRDAGH

SEQ ID NO: 79 - protein, 15 aa, synthetic construct
TVDGKRVPRDAGHPL

SEQ ID NO: 80 - protein, 9 aa, synthetic construct
YLMHWPYAF

SEQ ID NO: 81 - protein, 10 aa, synthetic construct
GESEAKVRIF

SEQ ID NO: 82 - protein, 9 aa, synthetic construct
HVYNYDFPR

SEQ ID NO: 83 - protein, 9 aa, synthetic construct
SAAEIYNEV